European Patent Application EP 4 136 963 A1, published February 22, 2023. Title: METHODS AND COMPOSITIONS FOR INCREASING EFFICIENCY OF TARGETED GENE MODIFICATION USING OLIGONUCLEOTIDE-MEDIATED GENE REPAIR. Applicant: CIBUS US LLC CIBUS EUROPE B.V. Application PCT/US2014/029566. The sequence listing filed with the application follows.

SEQUENCE LISTING (38 sequences)

SEQ ID NO: 1 - DNA, 99 bp, Artificial Sequence
  Description of Artificial Sequence: Synthetic oligonucleotide
  misc_feature (1)..(4): Phosphothioate linkage between nucleotides
  misc_feature (96)..(99): Phosphothioate linkage between nucleotides
gtcgtgctgcttcatgtggcggggtagcggctgaagcactgcacgccgtaggtgaaggtggtcacgagggtgggccaggcacgggcagcttgccggtgg

SEQ ID NO: 2 - DNA, 101 bp, Artificial Sequence
  Description of Artificial Sequence: Synthetic polynucleotide
  misc_feature (1)..(4): Phosphothioate linkage between nucleotides
  misc_feature (98)..(101): Phosphothioate linkage between nucleotides
gtcgtgctgcttcatgtggtcggggtagcggctgaagcactgcacgccgtgggtgaaggtggtcacgagggtgggccagggcacgggcagcttgccggtgg

SEQ ID NO: 3 - DNA, 101 bp, Artificial Sequence
  Description of Artificial Sequence: Synthetic polynucleotide
  misc_feature (1)..(4): Phosphothioate linkage between nucleotides
  misc_feature (98)..(101): Phosphothioate linkage between nucleotides
ccaccggcaagctgcccgtgccctggcccaccctcgtgaccaccttcacctacggcgtgcagtgcttcagccgctaccccgaccacatgaagcagcacgac

SEQ ID NO: 4 - DNA, 101 bp, Artificial Sequence
  Description of Artificial Sequence: Synthetic polynucleotide
  misc_feature (1)..(4): Phosphothioate linkage between nucleotides
  misc_feature (98)..(101): Phosphothioate linkage between nucleotides
ccaccggcaagctgcccgtgccctggcccaccctcgtgaccaccttcacccacggcgtgcagtgcttcagccgctaccccgaccacatgaagcagcacgac

SEQ ID NO: 5 - DNA, 201 bp, Artificial Sequence
  Description of Artificial Sequence: Synthetic polynucleotide
  misc_feature (1)..(4): Phosphothioate linkage between nucleotides
  misc_feature (198)..(201): Phosphothioate linkage between nucleotides
aagatggtgcgctcctggacgtagccttcgggcatggcggacttgaagaagtcgtgctgcttcatgtggtcggggtagcggctgaagcactgcacgccgtaggtgaaggtggtcacgagggtgggccagggcacgggcagcttgccggtggtgcagatgaacttcagggtcagcttgccgtaggtggcatcgccctcgccc

SEQ ID NO: 6 - DNA, 201 bp, Artificial Sequence
  Description of Artificial Sequence: Synthetic polynucleotide
  misc_feature (1)..(4): Phosphothioate linkage between nucleotides
  misc_feature (198)..(201): Phosphothioate linkage between nucleotides
aagatggtgcgctcctggacgtagccttcgggcatggcggacttgaagaagtcgtgctgcttcatgtggtcggggtagcggctgaagcactgcacgccgtgggtgaaggtggtcacgagggtgggccagggcacgggcagcttgccggtggtgcagatgaacttcagggtcagcttgccgtaggtggcatcgccctcgccc

SEQ ID NO: 7 - DNA, 201 bp, Artificial Sequence
  Description of Artificial Sequence: Synthetic polynucleotide
  misc_feature (1)..(4): Phosphothioate linkage between nucleotides
  misc_feature (198)..(201): Phosphothioate linkage between nucleotides
gggcgagggcgatgccacctacggcaagctgaccctgaagttcatctgcaccaccggcaagctgcccgtgccctggcccaccctcgtgaccaccttcacctacggcgtgcagtgcttcagccgctaccccgaccacatgaagcagcacgacttcttcaagtccgccatgcccgaaggctacgtccaggagcgcaccatctt

SEQ ID NO: 8 - DNA, 201 bp, Artificial Sequence
  Description of Artificial Sequence: Synthetic polynucleotide
  misc_feature (1)..(4): Phosphothioate linkage between nucleotides
  misc_feature (198)..(201): Phosphothioate linkage between nucleotides
gggcgagggcgatgccacctacggcaagctgaccctgaagttcatctgcaccaccggcaagctgcccgtgccctggcccaccctcgtgaccaccttcacccacggcgtgcagtgcttcagccgctaccccgaccacatgaagcagcacgacttcttcaagtccgccatgcccgaaggctacgtccaggagcgcaccatctt

SEQ ID NO: 9 - protein, 6 aa, Artificial Sequence
  Description of Artificial Sequence: Synthetic peptide
PKKRKV

SEQ ID NO: 10 - DNA, 110 bp, Artificial Sequence
  Description of Artificial Sequence: Synthetic polynucleotide
  modified_base (1)..(20): a, c, t, g, unknown or other
nnnnnnnnnnnnnnnnnnnngttttagagctagaaatagcaagttaaaataaggctagtccgttatgttcttgaaaaaagtgagtggcaccgagtcggtggtgctttttt

SEQ ID NO: 11 - RNA, 48 nt, Artificial Sequence
  Description of Artificial Sequence: Synthetic oligonucleotide
  modified_base (3)..(32): a, c, u, g, unknown or other
acnnnnnnnnnnnnnnnnnnnnnnnnnnnnnnguuuuagagcuaugcu

SEQ ID NO: 12 - DNA, 67 bp, Artificial Sequence
  Description of Artificial Sequence: Synthetic oligonucleotide
  Description of Combined DNA/RNA Molecule: Synthetic oligonucleotide
agcauagcaaguuaaaauaaggctaguccguuaucaacuugaaaaaguggcaccgagucggugcuuu

SEQ ID NO: 13 - RNA, 62 nt, Artificial Sequence
  Description of Artificial Sequence: Synthetic oligonucleotide
  modified_base (1)..(20): a, c, u, g, unknown or other
nnnnnnnnnnnnnnnnnnnnguuuuagagcuagaaauagcaaguuaaaauaaggcuaguccg

SEQ ID NO: 14 - DNA, 23 bp, Artificial Sequence
  Description of Artificial Sequence: Synthetic oligonucleotide
tcgtgaccaccttcacccacggc

SEQ ID NO: 15 - protein, 7 aa, Artificial Sequence
  Description of Artificial Sequence: Synthetic peptide
GVTTFTY

SEQ ID NO: 16 - DNA, 84 bp, Artificial Sequence
  Description of Artificial Sequence: Synthetic oligonucleotide
gtggaaaggacgaaacaccgggtcttcgagaagacctgttttagagctagaaatagcaagttaaaataaggctagtccgttttt

SEQ ID NO: 17 - DNA, 84 bp, Artificial Sequence
  Description of Artificial Sequence: Synthetic oligonucleotide
aaaaacggactagccttattttaacttgctatttctagctctaaaacaggtcttctcgaagacccggtgtttcgtcctttccac

SEQ ID NO: 18 - DNA, 24 bp, Artificial Sequence
  Description of Artificial Sequence: Synthetic oligonucleotide
  modified_base (6)..(24): a, c, t, g, unknown or other
caccgnnnnnnnnnnnnnnnnnnn

SEQ ID NO: 19 - DNA, 24 bp, Artificial Sequence
  Description of Artificial Sequence: Synthetic oligonucleotide
  modified_base (5)..(23): a, c, t, g, unknown or other
aaacnnnnnnnnnnnnnnnnnnnc

SEQ ID NO: 20 - protein, 11 aa, Artificial Sequence
  Description of Artificial Sequence: Synthetic peptide
TAMRPLTVAAV

SEQ ID NO: 21 - DNA, 41 bp, Artificial Sequence
  Description of Artificial Sequence: Synthetic oligonucleotide
actgcaatgcggccattgacagcagctgttactgctgctgg

SEQ ID NO: 22 - DNA, 20 bp, Artificial Sequence
  Description of Artificial Sequence: Synthetic oligonucleotide
ccgctgccgttactgctgca

SEQ ID NO: 23 - DNA, 20 bp, Artificial Sequence
  Description of Artificial Sequence: Synthetic oligonucleotide
cggctgcagttactgctgct

SEQ ID NO: 24 - DNA, 20 bp, Artificial Sequence
  Description of Artificial Sequence: Synthetic oligonucleotide
ccgctgcagttactgctgca

SEQ ID NO: 25 - DNA, 20 bp, Artificial Sequence
  Description of Artificial Sequence: Synthetic oligonucleotide
ccgctgcagttacagctgca

SEQ ID NO: 26 - DNA, 20 bp, Artificial Sequence
  Description of Artificial Sequence: Synthetic oligonucleotide
cagctgctgtaacagccgct

SEQ ID NO: 27 - DNA, 20 bp, Artificial Sequence
  Description of Artificial Sequence: Synthetic oligonucleotide
cagcagcagttgctgtagct

SEQ ID NO: 28 - DNA, 20 bp, Artificial Sequence
  Description of Artificial Sequence: Synthetic oligonucleotide
cagcagcagttacagtagct

SEQ ID NO: 29 - DNA, 20 bp, Artificial Sequence
  Description of Artificial Sequence: Synthetic oligonucleotide
tgcgcctcgctttgtcttgt

SEQ ID NO: 30 - DNA, 20 bp, Artificial Sequence
  Description of Artificial Sequence: Synthetic oligonucleotide
attttacaggtgtttacgcc

SEQ ID NO: 31 - DNA, 71 bp, Artificial Sequence
  Description of Artificial Sequence: Synthetic oligonucleotide
  Description of Combined DNA/RNA Molecule: Synthetic oligonucleotide
  modified_base (1)..(1): 2'-O-Me modified nucleotide
  modified_base (11)..(71): 2'-O-Me modified nucleotide
uucauguggucggggtagcggctgaagcactgcacgccgtaggtgaaggtggtcacgagggtgggccaggg

SEQ ID NO: 32 - DNA, 71 bp, Artificial Sequence
  Description of Artificial Sequence: Synthetic oligonucleotide
  Description of Combined DNA/RNA Molecule: Synthetic oligonucleotide
  modified_base (1)..(1): 2'-O-Me modified nucleotide
  modified_base (11)..(71): 2'-O-Me modified nucleotide
uucauguggucggggtagcggctgaagcactgcacgccgtgggtgaaggtggtcacgagggtgggccaggg

SEQ ID NO: 33 - DNA, 71 bp, Artificial Sequence
  Description of Artificial Sequence: Synthetic oligonucleotide
  Description of Combined DNA/RNA Molecule: Synthetic oligonucleotide
  modified_base (1)..(1): 2'-O-Me modified nucleotide
  modified_base (11)..(71): 2'-O-Me modified nucleotide
gcugcccgugccctggcccaccctcgtgaccaccttcacctacggcgtgcagtgcttcagccgctaccccg

SEQ ID NO: 34 - DNA, 71 bp, Artificial Sequence
  Description of Artificial Sequence: Synthetic oligonucleotide
  Description of Combined DNA/RNA Molecule: Synthetic oligonucleotide
  modified_base (1)..(1): 2'-O-Me modified nucleotide
  modified_base (11)..(71): 2'-O-Me modified nucleotide
gcugcccgugccctggcccaccctcgtgaccaccttcacccacggcgtgcagtgcttcagccgctaccccg

SEQ ID NO: 35 - DNA, 71 bp, Artificial Sequence; identical to SEQ ID NO: 31
  Description of Artificial Sequence: Synthetic oligonucleotide
  Description of Combined DNA/RNA Molecule: Synthetic oligonucleotide
  modified_base (1)..(9): 2'-O-Me modified nucleotide
  modified_base (11)..(71): 2'-O-Me modified nucleotide

SEQ ID NO: 36 - DNA, 71 bp, Artificial Sequence; identical to SEQ ID NO: 32
  Description of Artificial Sequence: Synthetic oligonucleotide
  Description of Combined DNA/RNA Molecule: Synthetic oligonucleotide
  modified_base (1)..(9): 2'-O-Me modified nucleotide
  modified_base (11)..(71): 2'-O-Me modified nucleotide

SEQ ID NO: 37 - DNA, 71 bp, Artificial Sequence; identical to SEQ ID NO: 33
  Description of Artificial Sequence: Synthetic oligonucleotide
  Description of Combined DNA/RNA Molecule: Synthetic oligonucleotide
  modified_base (1)..(9): 2'-O-Me modified nucleotide
  modified_base (11)..(71): 2'-O-Me modified nucleotide

SEQ ID NO: 38 - DNA, 71 bp, Artificial Sequence; identical to SEQ ID NO: 34
  Description of Artificial Sequence: Synthetic oligonucleotide
  Description of Combined DNA/RNA Molecule: Synthetic oligonucleotide
  modified_base (1)..(9): 2'-O-Me modified nucleotide
  modified_base (11)..(71): 2'-O-Me modified nucleotide